European Patent Application EP 4 707 386 A1, published March 11, 2026. Title: ARTIFICIAL VIRUS CAPSID. Applicant: AGC Inc. Application WO. The sequence listing filed with the application follows.

SEQUENCE LISTING (3 sequences)

SEQ ID NO: 1 - protein, 24 aa, tomato bushy stunt virus
INHVGGTGGAIMAPVAVTRQLVGS

SEQ ID NO: 2 - protein, 24 aa, synthetic construct
INHVGGTGGAIMAPVAVTRQLVCS

SEQ ID NO: 3 - protein, 24 aa, synthetic construct
INHVGGTGGAIMAPVAVTRQLVGC